European Patent Specification EP 3 898 955 B1, published March 22, 2023. Title: DNA aptamers specific of Adenovirus types. Applicant: Luxembourg Institute of Science and Technology (LIST). The sequence listing filed with the application follows.

SEQUENCE LISTING (5 sequences)

SEQ ID NO: 1 - DNA, 65 bp, Artificial sequence
  Aptamer specific of Adenoviruses
gtgccagctatgccattgggggacaatatcgcagtgcatcttcctctagcgtctatctctgctgc

SEQ ID NO: 2 - DNA, 65 bp, Artificial sequence
  Aptamer specific of Adenoviruses
gtgccagctatgccattggccagtagtttcagtctaccaacggtcatagcgtctatctctgctgc

SEQ ID NO: 3 - DNA, 65 bp, Artificial sequence
  Aptamer specific of Adenoviruses
gtgccagctatgccattgggcgggtcgtccaattcgagaggtcccctagcgtctatctctgctgc

SEQ ID NO: 4 - DNA, 18 bp, Artificial sequence
  Oligonucleotide primer
gtgccagctatgccattg

SEQ ID NO: 5 - DNA, 19 bp, Artificial sequence
  Oligonucleotide primer
gcagcagagatagacgcta